European Patent Application EP 4 145 132 A1, published March 8, 2023. Title: METHODS AND KIT FOR DETERMINING THE ANTIBODY STATUS AND T-CELL IMMUNITY AGAINST SARS-CoV-2. Applicant: ISAR Bioscience GmbH. The sequence listing filed with the application follows.

SEQUENCE LISTING (7 sequences)

SEQ ID NO: 1 - protein, 224 aa, artificial sequence
  wild type SARS-CoV-2 RBD
MRVQPTESIVRFPNITNLCPFGEVFNATRFASVYAWNRKRISNCVADYSVLYNSASFSTFKCYGVSPTKLNDLCFTNVYADSFVIRGDEVRQIAPGQTGKIADYNYKLPDDFTGCVIAWNSNNLDSKVGGNYNYLYRLFRKSNLKPFERDISTEIYQAGSTPCNGVEGFNCYFPLQSYGFQPTNGVGYQPYRVVVLSFELLHAPATVCGPKKSTNLVKNKCVNF

SEQ ID NO: 2 - protein, 224 aa, Artificial Sequence
  alpha SARS-CoV-2 RBD
MRVQPTESIVRFPNITNLCPFGEVFNATRFASVYAWNRKRISNCVADYSVLYNSASFSTFKCYGVSPTKLNDLCFTNVYADSFVIRGDEVRQIAPGQTGKIADYNYKLPDDFTGCVIAWNSNNLDSKVGGNYNYLYRLFRKSNLKPFERDISTEIYQAGSTPCNGVEGFNCYFPLQSYGFQPTYGVGYQPYRVVVLSFELLHAPATVCGPKKSTNLVKNKCVNF

SEQ ID NO: 3 - protein, 224 aa, Artificial Sequence
  beta SARS-CoV-2 RBD
MRVQPTESIVRFPNITNLCPFGEVFNATRFASVYAWNRKRISNCVADYSVLYNSASFSTFKCYGVSPTKLNDLCFTNVYADSFVIRGDEVRQIAPGQTGNIADYNYKLPDDFTGCVIAWNSNNLDSKVGGNYNYLYRLFRKSNLKPFERDISTEIYQAGSTPCNGVKGFNCYFPLQSYGFQPTYGVGYQPYRVVVLSFELLHAPATVCGPKKSTNLVKNKCVNF

SEQ ID NO: 4 - protein, 224 aa, Artificial Sequence
  gamma SARS-Cov-2 RBD
MRVQPTESIVRFPNITNLCPFGEVFNATRFASVYAWNRKRISNCVADYSVLYNSASFSTFKCYGVSPTKLNDLCFTNVYADSFVIRGDEVRQIAPGQTGTIADYNYKLPDDFTGCVIAWNSNNLDSKVGGNYNYLYRLFRKSNLKPFERDISTEIYQAGSTPCNGVKGFNCYFPLQSYGFQPTYGVGYQPYRVVVLSFELLHAPATVCGPKKSTNLVKNKCVNF

SEQ ID NO: 5 - protein, 224 aa, Artificial Sequence
  delta SARS-CoV-2 RBD
MRVQPTESIVRFPNITNLCPFGEVFNATRFASVYAWNRKRISNCVADYSVLYNSASFSTFKCYGVSPTKLNDLCFTNVYADSFVIRGDEVRQIAPGQTGKIADYNYKLPDDFTGCVIAWNSNNLDSKVGGNYNYRYRLFRKSNLKPFERDISTEIYQAGSKPCNGVEGFNCYFPLQSYGFQPTNGVGYQPYRVVVLSFELLHAPATVCGPKKSTNLVKNKCVNF

SEQ ID NO: 6 - protein, 230 aa, Artificial Sequence
  wt RBD with C-terminal His-tag of the S protein of wt SARS-CoV-2
MRVQPTESIVRFPNITNLCPFGEVFNATRFASVYAWNRKRISNCVADYSVLYNSASFSTFKCYGVSPTKLNDLCFTNVYADSFVIRGDEVRQIAPGQTGKIADYNYKLPDDFTGCVIAWNSNNLDSKVGGNYNYLYRLFRKSNLKPFERDISTEIYQAGSTPCNGVEGFNCYFPLQSYGFQPTNGVGYQPYRVVVLSFELLHAPATVCGPKKSTNLVKNKCVNFHHHHHH

SEQ ID NO: 7 - protein, 249 aa, Artificial Sequence
  wt RBD with N-terminal signal sequence and C-terminal His-tag of the S protein of wt SARS-CoV-2
METPAQLLFLLLLWLPDTTGRVQPTESIVRFPNITNLCPFGEVFNATRFASVYAWNRKRISNCVADYSVLYNSASFSTFKCYGVSPTKLNDLCFTNVYADSFVIRGDEVRQIAPGQTGKIADYNYKLPDDFTGCVIAWNSNNLDSKVGGNYNYLYRLFRKSNLKPFERDISTEIYQAGSTPCNGVEGFNCYFPLQSYGFQPTYGVGYQPYRVVVLSFELLHAPATVCGPKKSTNLVKNKCVNFHHHHHH